European Patent Application EP 4 799 609 A1, published September 2, 2026. Title: 펩타이드 함유 액상제제 및 그 제조방법. Applicant: 주식회사 엔솔바이오사이언스. Application KR. The sequence listing filed with the application follows.

SEQUENCE LISTING (1 sequence)

SEQ ID NO: 1 - protein, 5 aa, synthetic construct
ELHLD